European Patent Application EP 4 706 677 A1, published March 11, 2026. Title: THERAPEUTIC EFFECT ENHANCER FOR ENHANCING EFFECT OF CAR-T THERAPY. Applicant: Kabishiki Kaisya Toshiba. Application EP. The sequence listing filed with the application follows.

SEQUENCE LISTING (4 sequences)

SEQ ID NO: 1 - protein, 20 aa, synthetic construct
  REGION 1..20: note = Nucleic acid condensing peptide
RQRQRYYRQRQRGGRRRRRR

SEQ ID NO: 2 - protein, 13 aa, synthetic construct
  REGION 1..13: note = Nucleic acid condensing peptide
RQRQRGGRRRRRR

SEQ ID NO: 3 - protein, 21 aa, synthetic construct
  REGION 1..21: note = Nucleic acid condensing peptide
RRRRRRYYRQRQRGGRRRRRR

SEQ ID NO: 4 - protein, 39 aa, Homo sapiens
GNQSSNFGPMKGGNFGGRSSGPYGGGGQYFAKPRNQGGY